European Patent Application EP 4 230 723 A1, published August 23, 2023. Title: 具有天冬氨酸激酶活性的多肽及其在生产氨基酸中的应用. Applicant: 中国科学院天津工业生物技术研究所. The sequence listing filed with the application follows.

SEQUENCE LISTING (50 sequences)

SEQ ID NO: 1 - protein, 421 aa, Corynebacterium glutamicum
MALVVQKYGGSSLESAERIRNVAERIVATKKAGNDVVVVCSAMGDTTDELLELAAAVNPVPPAREMDMLLTAGERISNALVAMAIESLGAEAQSFTGSQAGVLTTERHGNARIVDVTPGRVREALDEGKICIVAGFQGVNKETRDVTTLGRGGSDTTAVALAAALNADVCEIYSDVDGVYTADPRIVPNAQKLEKLSFEEMLELAAVGSKILVLRSVEYARAFNVPLRVRSSYSNDPGTLIAGSMEDIPVEEAVLTGVATDKSEAKVTVLGISDKPGEAAKVFRALADAEINIDMVLQNVSSVEDGTTDITFTCPRSDGRRAMEILKKLQVQGNWTNVLYDDQVGKVSLVGAGMKSHPGVTAEFMEALRDVNVNIELISTSEIRISVLIREDDLDAAARALHEQFQLGGEDEAVVYAGTGR

SEQ ID NO: 2 - DNA, 1266 bp, Artificial Sequence
  LysC基因序列
gtggccctggtcgtacagaaatatggcggttcctcgcttgagagtgcggaacgcattagaaacgtcgctgaacggatcgttgccaccaagaaggctggaaatgatgtcgtggttgtctgctccgcaatgggagacaccacggatgaacttctagaacttgcagcggcagtgaatcccgttccgccagctcgtgaaatggatatgctcctgactgctggtgagcgtatttctaacgctctcgtcgccatggctattgagtcccttggcgcagaagcccaatctttcacgggctctcaggctggtgtgctcaccaccgagcgccacggaaacgcacgcattgttgatgtcactccaggtcgtgtgcgtgaagcactcgatgagggcaagatctgcattgttgctggtttccagggtgttaataaagaaacccgcgatgtcaccacgttgggtcgtggtggttctgacaccactgcagttgcgttggcagctgctttgaacgctgatgtgtgtgagatttactcggacgttgacggtgtgtataccgctgacccgcgcatcgttcctaatgcacagaagctggaaaagctcagcttcgaagaaatgctggaacttgctgctgttggctccaagattttggtgctgcgcagtgttgaatacgctcgtgcattcaatgtgccacttcgcgtacgctcgtcttatagtaatgatcccggcactttgattgccggctctatggaggatattcctgtggaagaagcagtccttaccggtgtcgcaaccgacaagtccgaagccaaagtaaccgttctgggtatttccgataagccaggcgaggctgcgaaggttttccgtgcgttggctgatgcagaaatcaacattgacatggttctgcagaacgtctcttctgtagaagacggcaccaccgacatcaccttcacctgccctcgttccgacggccgccgcgcgatggagatcttgaagaagcttcaggttcagggcaactggaccaatgtgctttacgacgaccaggtcggcaaagtctccctcgtgggtgctggcatgaagtctcacccaggtgttaccgcagagttcatggaagctctgcgcgatgtcaacgtgaacatcgaattgatttccacctctgagattcgtatttccgtgctgatccgtgaagatgatctggatgctgctgcacgtgcattgcatgagcagttccagctgggcggcgaagacgaagccgtcgtttatgcaggcaccggacgctaa

SEQ ID NO: 3 - DNA, 11773 bp, Artificial Sequence
  质粒序列
aattaagcttaaaggcacccgatatggataagaaatactcaataggcttagatatcggcacaaatagcgtcggatgggcggtgatcactgatgaatataaggttccgtctaaaaagttcaaggttctgggaaatacagaccgccacagtatcaaaaaaaatcttataggggctcttttatttgacagtggagagacagcggaagcgactcgtctcaaacggacagctcgtagaaggtatacacgtcggaagaatcgtatttgttatctacaggagattttttcaaatgagatggcgaaagtagatgatagtttctttcatcgacttgaagagtcttttttggtggaagaagacaagaagcatgaacgtcatcctatttttggaaatatagtagatgaagttgcttatcatgagaaatatccaactatctatcatctgcgaaaaaaattggtagattctactgataaagcggatttgcgcttaatctatttggccttagcgcatatgattaagtttcgtggtcattttttgattgagggagatttaaatcctgataatagtgatgtggacaaactatttatccagttggtacaaacctacaatcaattatttgaagaaaaccctattaacgcaagtggagtagatgctaaagcgattctttctgcacgattgagtaaatcaagacgattagaaaatctcattgctcagctccccggtgagaagaaaaatggcttatttgggaatctcattgctttgtcattgggtttgacccctaattttaaatcaaattttgatttggcagaagatgctaaattacagctttcaaaagatacttacgatgatgatttagataatttattggcgcaaattggagatcaatatgctgatttgtttttggcagctaagaatttatcagatgctattttactttcagatatcctaagagtaaatactgaaataactaaggctcccctatcagcttcaatgattaaacgctacgatgaacatcatcaagacttgactcttttaaaagctttagttcgacaacaacttccagaaaagtataaagaaatcttttttgatcaatcaaaaaacggatatgcaggttatattgatgggggagctagccaagaagaattttataaatttatcaaaccaattttagaaaaaatggatggtactgaggaattattggtgaaactaaatcgtgaagatttgctgcgcaagcaacggacctttgacaacggctctattccccatcaaattcacttgggtgagctgcatgctattttgagaagacaagaagacttttatccatttttaaaagacaatcgtgagaagattgaaaaaatcttgacttttcgaattccttattatgttggtccattggcgcgtggcaatagtcgttttgcatggatgactcggaagtctgaagaaacaattaccccatggaattttgaagaagttgtcgataaaggtgcttcagctcaatcatttattgaacgcatgacaaactttgataaaaatcttccaaatgaaaaagtactaccaaaacatagtttgctttatgagtattttacggtttataacgaattgacaaaggtcaaatatgttactgaaggaatgcgaaaaccagcatttctttcaggtgaacagaagaaagccattgttgatttactcttcaaaacaaatcgaaaagtaaccgttaagcaattaaaagaagattatttcaaaaaaatagaatgttttgatagtgttgaaatttcaggagttgaagatagatttaatgcttcattaggtacctaccatgatttgctaaaaattattaaagataaagattttttggataatgaagaaaatgaagatatcttagaggatattgttttaacattgaccttatttgaagatagggagatgattgaggaaagacttaaaacatatgctcacctctttgatgataaggtgatgaaacagcttaaacgtcgccgttatactggttggggacgtttgtctcgaaaattgattaatggtattagggataagcaatctggcaaaacaatattagattttttgaaatcagatggttttgccaatcgcaattttatgcagctgatccatgatgatagtttgacatttaaagaagacattcaaaaagcacaagtgtctggacaaggcgatagtttacatgaacatattgcaaatttagctggtagccctgctattaaaaaaggtattttacagactgtaaaagttgttgatgaattggtcaaagtaatggggcggcataagccagaaaatatcgttattgaaatggcacgtgaaaatcagacaactcaaaagggccagaaaaattcgcgagagcgtatgaaacgaatcgaagaaggtatcaaagaattaggaagtcagattcttaaagagcatcctgttgaaaatactcaattgcaaaatgaaaagctctatctctattatctccaaaatggaagagacatgtatgtggaccaagaattagatattaatcgtttaagtgattatgatgtcgatcacattgttccacaaagtttccttaaagacgattcaatagacaataaggtcttaacgcgttctgataaaaatcgtggtaaatcggataacgttccaagtgaagaagtagtcaaaaagatgaaaaactattggagacaacttctaaacgccaagttaatcactcaacgtaagtttgataatttaacgaaagctgaacgtggaggtttgagtgaacttgataaagctggttttatcaaacgccaattggttgaaactcgccaaatcactaagcatgtggcacaaattttggatagtcgcatgaatactaaatacgatgaaaatgataaacttattcgagaggttaaagtgattaccttaaaatctaaattagtttctgacttccgaaaagatttccaattctataaagtacgtgagattaacaattaccatcatgcccatgatgcgtatctaaatgccgtcgttggaactgctttgattaagaaatatccaaaacttgaatcggagtttgtctatggtgattataaagtttatgatgttcgtaaaatgattgctaagtctgagcaagaaataggcaaagcaaccgcaaaatatttcttttactctaatatcatgaacttcttcaaaacagaaattacacttgcaaatggagagattcgcaaacgccctctaatcgaaactaatggggaaactggagaaattgtctgggataaagggcgagattttgccacagtgcgcaaagtattgtccatgccccaagtcaatattgtcaagaaaacagaagtacagacaggcggattctccaaggagtcaattttaccaaaaagaaattcggacaagcttattgctcgtaaaaaagactgggatccaaaaaaatatggtggttttgatagtccaacggtagcttattcagtcctagtggttgctaaggtggaaaaagggaaatcgaagaagttaaaatccgttaaagagttactagggatcacaattatggaaagaagttcctttgaaaaaaatccgattgactttttagaagctaaaggatataaggaagttaaaaaagacttaatcattaaactacctaaatatagtctttttgagttagaaaacggtcgtaaacggatgctggctagtgccggagaattacaaaaaggaaatgagctggctctgccaagcaaatatgtgaattttttatatttagctagtcattatgaaaagttgaagggtagtccagaagataacgaacaaaaacaattgtttgtggagcagcataagcattatttagatgagattattgagcaaatcagtgaattttctaagcgtgttattttagcagatgccaatttagataaagttcttagtgcatataacaaacatagagacaaaccaatacgtgaacaagcagaaaatattattcatttatttacgttgacgaatcttggagctcccgctgcttttaaatattttgatacaacaattgatcgtaaacgatatacgtctacaaaagaagttttagatgccactcttatccatcaatccatcactggtctttatgaaacacgcattgatttgagtcagctaggaggtgactgaagcttggctgttttggcggatgagagaagattttcagcctgatacagattaaatcagaacgcagaagcggtctgataaaacagaatttgcctggcggcagtagcgcggtggtcccacctgaccccatgccgaactcagaagtgaaacgccgtagcgccgatggtagtgtggggtctgcccatgcgagagtagggaactgccaggcatcaaataaaacgaaaggctcagtcgaaagactgggcctttcgttttatctgttgtttgtcggtgaacgctctcctgagtaggacaaatccgccgggagcggatttgaacgttgcgaagcaacggcccggagggtggcgggcaggacgcccgccataaactgccaggcatcaaattaagcagaaggccatcctgacggatggcctttttgcgtttctacaaactcttttgtttatttttctaaatacattcaaatatgtatccgctcatgagacaataaccctgataaatgcttcaataatattgaaaaaggaagagtatgagtattcaacatttccgtgtcgcccttattcccttttttgcggcattttgccttcctgtttttgctcacccagaaacgctggtgaaagtaaaagatgctgaagatcagttgggtgcacgagtgggttacatcgaactggatctcaacagcggtaagatccttgagagttttcgccccgaagaacgttttccaatgatgagcacttttgcttcctcgctcactgactcgctgcgctcggtcgttcggctgcggcgagcggtatcagctcactcaaaggcggtaatacggttatccacagaatcaggggataacgcaggaaagaacatgtgagcaaaaggccagcaaaaggccaggaaccgtaaaaaggccgcgttgctggcgtttttccataggctccgcccccctgacgagcatcacaaaaatcgacgctcaagtcagaggtggcgaaacccgacaggactataaagataccaggcgtttccccctggaagctccctcgtgcgctctcctgttccgaccctgccgcttaccggatacctgtccgcctttctcccttcgggaagcgtggcgctttctcaatgctcacgctgtaggtatctcagttcggtgtaggtcgttcgctccaagctgggctgtgtgcacgaaccccccgttcagcccgaccgctgcgccttatccggtaactatcgtcttgagtccaacccggtaagacacgacttatcgccactggcagcagccactggtaacaggattagcagagcgaggtatgtaggcggtgctacagagttcttgaagtggtggcctaactacggctacactagaaggacagtatttggtatctgcgctctgctgaagccagttaccttcggaaaaagagttggtagctcttgatccggcaaacaaaccaccgctggtagcggtggtttttttgtttgcaagcagcagattacgcgcagaaaaaaaggatctcaagaagatcctttgatcttttctacggggtctgacgctcagtggaacgaaaactcacgttaagggattttggtcatgagattatcaaaaaggatcttcacctagatccttttggggtgggcgaagaactccagcatgagatccccgcgctggaggatcatccagccattcggggtcgttcactggttcccctttctgatttctggcatagaagaacccccgtgaactgtgtggttccgggggttgctgatttttgcgagacttctcgcgcaattccctagcttaggtgaaaacaccatgaaacactagggaaacacccatgaaacacccattagggcagtagggcggcttcttcgtctagggcttgcatttgggcggtgatctggtctttagcgtgtgaaagtgtgtcgtaggtggcgtgctcaatgcactcgaacgtcacgtcatttaccgggtcacggtgggcaaagagaactagtgggttagacattgttttcctcgttgtcggtggtggtgagcttttctagccgctcggtaaacgcggcgatcatgaactcttggaggttttcaccgttctgcatgcctgcgcgcttcatgtcctcacgtagtgccaaaggaacgcgtgcggtgaccacgacgggcttagcctttgcctgcgcttctagtgcttcgatggtggcttgtgcctgcgcttgctgcgcctgtagtgcctgttgagcttcttgtagttgctgttctagctgtgccttggttgccatgctttaagactctagtagctttcctgcgatatgtcatgcgcatgcgtagcaaacattgtcctgcaactcattcattatgtgcagtgctcctgttactagtcgtacatactcatatttacctagtctgcatgcagtgcatgcacatgcagtcatgtcgtgctaatgtgtaaaacatgtacatgcagattgctgggggtgcagggggcggagccaccctgtccatgcggggtgtggggcttgccccgccggtacagacagtgagcaccggggcacctagtcgcggataccccccctaggtatcggacacgtaaccctcccatgtcgatgcaaatctttaacattgagtacgggtaagctggcacgcatagccaagctaggcggccaccaaacaccactaaaaattaatagtccctagacaagacaaacccccgtgcgagctaccaactcatatgcacgggggccacataacccgaaggggtttcaattgacaaccatagcactagctaagacaacgggcacaacacccgcacaaactcgcactgcgcaaccccgcacaacatcgggtctaggtaacactgagtaacactgaaatagaagtgaacacctctaaggaaccgcaggtcaatgagggttctaaggtcactcgcgctagggcgtggcgtaggcaaaacgtcatgtacaagatcaccaatagtaaggctctggcggggtgccataggtggcgcagggacgaagctgttgcggtgtcctggtcgtctaacggtgcttcgcagtttgagggtctgcaaaactctcactctcgctgggggtcatctctggctgaattggaagtcatgggcgaacgccgcattgagctggctattgctactaagaatcacttggcggcgggtggcgcgctcatgatgtttgtgggcactgttcgacacaaccgctcacagtcatttgcgcaggttgaagcgggtattaagactgcgtactcttcgatggtgaaaacatctcagtggaagaaagaacgtgcacggtacggggtggagcacacctatagtgactatgaggtcacagactcttgggcgaacggttggcacttgcaccgcaacatgctgttgttcttggatcgtccactgtctgacgatgaactcaaggcgtttgaggattccatgttttcccgctggtctgctggtgtggttaaggccggtatggacgcgccactgcgtgagcacggggtcaaacttgatcaggtgtctacctggggtggagacgctgcgaaaatggcaacctacctcgctaagggcatgtctcaggaactgactggctccgctactaaaaccgcgtctaaggggtcgtacacgccgtttcagatgttggatatgttggccgatcaaagcgacgccggcgaggatatggacgctgttttggtggctcggtggcgtgagtatgaggttggttctaaaaacctgcgttcgtcctggtcacgtggggctaagcgtgctttgggcattgattacatagacgctgatgtacgtcgtgaaatggaagaagaactgtacaagctcgccggtctggaagcaccggaacgggtcgaatcaacccgcgttgctgttgctttggtgaagcccgatgattggaaactgattcagtctgatttcgcggttaggcagtacgttctcgattgcgtggataaggctaaggacgtggccgctgcgcaacgtgtcgctaatgaggtgctggcaagtctgggtgtggattccaccccgtgcatgatcgttatggatgatgtggacttggacgcggttctgcctactcatggggacgctactaagcgtgatctgaatgcggcggtgttcgcgggtaatgagcagactattcttcgcacccactaaaagcggcataaaccccgttcgatattttgtgcgatgaatttatggtcaatgtcgcgggggcaaactatgatgggtcttgttgttggcgtcccggaaaacgattccgaagcccaacctttcatagaaggcggcggtggaatttttctccacataagctggcaatgttgcgacgcaacaggtacagtgtaattcatgagaccacgcgtggatccggcttactaaaagccagataacagtatgcgtatttgcgcgctgatttttgcggtataagaatatatactgatatgtatacccgaagtatgtcaaaaagaggtatgctatgaagcagcgtattacagtgacagttgacagcgacagctatcagttgctcaaggcatatatgatgtcaatatctccggtctggtaagcacaaccatgcagaatgaagcccgtcgtctgcgtgccgaacgctggaaagcggaaaatcaggaagggatggctgaggtcgcccggtttattgaaatgaacggctcttttgctgacgagaacaggggctggtgaaatgcagtttaaggtttacacctataaaagagagagccgttatcgtctgtttgtggatgtacagagtgatattattgacacgcccgggcgacggatggtgatccccctggccagtgcacgtctgctgtcagataaagtctcccgtgaactttacccggtggtgcatatcggggatgaaagctggcgcatgatgaccaccgatatggccagtgtgccggtatccgttatcggggaagaagtggctgatctcagccaccgcgaaaatgacatcaaaaacgccattaacctgatgttctggggaatataaggtctcagttttagagctagaaatagcaagttaaaataaggctagtccgttatcaacttgaaaaagtggcaccgagtcggtgctttttttccaggcatcaaataaaacgaaaggctcagtcgaaagactgggcctttcgttttatctgttgtttgtcggtgaacgctctcctgagtaggacaaatccgccgggagcggatttgaacgttgcgaagcaacggcccggagggtggcgggcaggacgcccgccataaactgccaggcatcaaattaagcagaaggccatcctgacggatggcctttttgcgtttctacaaactctttttgtttatttttctaaatacattcaaatatgtatccgctcatgaattaattccgctagatgacgtgcggcttcgaaaatctcgtgatggcaggttgggcgtcgcttggtcggtcatttcgaagggcaccaataactgccttaaaaaaattacgccccgccctgccactcatcgcagtactgttgtaattcattaagcattctgccgacatggaagccatcacagacggcatgatgaacctgaatcgccagcggcatcagcaccttgtcgccttgcgtataatatttgcccatggtgaaaacgggggcgaagaagttgtccatattggccacgtttaaatcaaaactggtgaaactcacccagggattggctgagacgaaaaacatattctcaataaaccctttagggaaataggccaggttttcaccgtaacacgccacatcttgcgaatatatgtgtagaaactgccggaaatcgtcgtggtattcactccagagcgatgaaaacgtttcagtttgctcatggaaaacggtgtaacaagggtgaacactatcccatatcaccagctcaccgtctttcattgccatacggaactccggatgagcattcatcaggcgggcaagaatgtgaataaaggccggataaaacttgtgcttatttttctttacggtctttaaaaaggccgtaatatccagctgaacggtctggttataggtacattgagcaactgactgaaatgcctcaaaatgttctttacgatgccattgggatatatcaacggtggtatatccagtgatttttttctccattttagcttccttagctcctgaaaatctcgtcgaagctcggcggatttgtcctactcaagctgatccgacaaaatccacacattatcccaggtgtccggatcggtcaaatacgctgccagctcatagaccgtatccaaagcatccggggctgatccccggcgccagggtggtttttcttttcaccagtgagacgggcaacagctgattgcccttcaccgcctggccctgagagagttgcagcaagcggtccacgtggtttgccccagcaggcgaaaatcctgtttgatggtggttaacggcgggatataacatgagctgtcttcggtatcgtcgtatcccactaccgagatatccgcaccaacgcgcagcccggactcggtaatggcgcgcattgcgcccagcgccatctgatcgttggcaaccagcatcgcagtgggaacgatgccctcattcagcatttgcatggtttgttgaaaaccggacatggcactccagtcgccttcccgttccgctatcggctgaatttgattgcgagtgagatatttatgccagccagccagacgcagacgcgccgagacagaacttaatgggcccgctaacagcgcgatttgctggtgacccaatgcgaccagatgctccacgcccagtcgcgtaccgtcttcatgggagaaaataatactgttgatgggtgtctggtcagagacatcaagaaataacgccggaacattagtgcaggcagcttccacagcaatggcatcctggtcatccagcggatagttaatgatcagcccactgacgcgttgcgcgagaagattgtgcaccgccgctttacaggcttcgacgccgcttcgttctaccatcgacaccaccacgctggcacccagttgatcggcgcgagatttaatcgccgcgacaatttgcgacggcgcgtgcagggccagactggaggtggcaacgccaatcagcaacgactgtttgcccgccagttgttgtgccacgcggttgggaatgtaattcagctccgccatcgccgcttccactttttcccgcgttttcgcagaaacgtggctggcctggttcaccacgcgggaaacggtctgataagagacaccggcatactctgcgacatcgtataacgttactggtttcacattcaccaccctgaattgactctcttccgggcgctatcatgccataccgcgaaaggttttgcaccattcgatggtgtcaacgtaaatgccgcttcgccttcgcgcgcgaattgcaagctgatccgggcttatcgactgcacggtgcaccaatgcttctggcgtcaggcagccatcggaagctgtggtatggctgtgcaggtcgtaaatcactgcataattcgtgtcgctcaaggcgcactcccgttctggataatgttttttgcgccgacatcataacggttctggcaaatattctgaaatgagctgttgacaattaatcatcggctcgtataatgtgtggaattgtgagcgctcacaatttcacacaggaaacagaatt

SEQ ID NO: 4 - DNA, 351 bp, Corynebacterium glutamicum
  ddh基因的启动子突变体序列
gtgcgtggcgagttttacaaagaaccccacatcatcaatgcctaaatggcgggtattttcatccaaacccaaccgcgcatcattccaatgctgatccaccccatccggataaaccaccatgaacggcaacggatcaaaagtcctgttggtgaagctgcgccccacagatcctgactgctgggagccatgaaaatagatcagcgcatccgtggtggaaccaaaaggctcaacaatacgaaacgttcgctttcggtcctgatgaaagagatgtccctgaatcatcatctaagtacaaaaggtggtaagctcgaccaggacagtgccaccacaattttggaggattacaagaac

SEQ ID NO: 5 - DNA, 5688 bp, Artificial Sequence
  质粒序列
gtgcgtggcgagttttacaaagaaccccacatcatcaatgcctaaatggcgggtattttcatccaaacccaaccgcgcatcattccaatgctgatccaccccatccggataaaccaccatgaacggcaacggatcaaaagtcctgttggtgaagctgcgccccacagatcctgactgctgggagccatgaaaatagatcagcgcatccgtggtggaaccaaaaggctcaacaatacgaaacgttcgctttcggtcctgatgaaagagatgtccctgaatcatcatctaagtacaaaaggtggtaagctcgaccaggacagtgccaccacaattttggaggattacaagaacatgactaagcaaccaccaatcgcaaaagccgatctgcaaaaaactcagggaaaccgtgcaccagcagcagttaaaaatagcgacgtgattagttttattaaccagccatcaatgaaagagcaactggcagcagctcttccacgccatatgacggctgaacgtatgatccgtatcgccaccacagaaattcgtaaagttccggcgttaggaaactgtgacactatgagttttgtcagtgcgatcgtacagtgttcacagctcggacttgagccaggtagcgccctcggtcatgcatatttactgccttttggtaataaaaacgaaaagagcggtaaaaagaacgttcagctaatcattggctatcgcggcatgattgatctggctcgccgttctggtcaaatcgccagcctgtcagcccgtgttgtccgtgaaggtgacgagtttagcttcgaatttggccttgatgaaaagttaatacaccgcccgggagaaaacgaagatgccccggttacccacgtctatgctgtcgcaagactgaaagacggaggtactcagtttgaagttatgacgcgcaaacagattgagctggtgcgcagcctgagtaaagctggtaataacgggccgtgggtaactcactgggaagaaatggcaaagaaaacggctattcgtcgcctgttcaaatatttgcccgtatcaattgagatccagcgtgcagtatcaatggatgaaaaggaaccactgacaatcgatcctgcagattcctctgtattaaccggggaatacagtgtaatcgataattcagaggaataactgttttggcggatgagagaagattttcagcctgatacagattaaatcagaacgcagaagcggtctgataaaacagaatttgcctggcggcagtagcgcggtggtcccacctgaccccatgccgaactcagaagtgaaacgccgtagcgccgatggtagtgtggggtctccccatgcgagagtagggaactgccaggcatcaaataaaacgaaaggctcagtcgaaagactgggcctttcgttttatctgttgtttgtcggtgaacgctctcctgagtaggacaaatccgccgggagcggatttgaacgttgcgaagcaacggcccggagggtggcgggcaggacgcccgccataaactgccaggcatcaaattaagcagaaggccatcctgacggatggcctttttgcgtttctacaaactctttttgtttatttttctaaatacattcaaatatgtatccgctcatgaattaattccgctagatgacgtgcggcttcgactagctccaaaaaggtctccaggatctcgaggagatttttgagggggagggagtcgaggaagagccagagcagaaggcggggaaccgttctctgccgacagcgtgagccccccttaaaaatcaggccggggaggaaccggggagggatcagagctaggagcgagacaccctaaagggggggaaccgttttctgctgacggtgtttcgtttattagttttcagcccgtggatagcggagggtgagggcaagtgagagccagagcaaggacgggacccctaaaggggggaaccgttttctgctgacggtgtttcgtttattagttttcagcccgtggacggccgcgtttagcttccattccaagtgcctttctgacttgttggatgcgcctttcactgacacctagttcgcctgcaagctcacgagtcgagggatcagcaaccgattgagaacgggcatccaggatcgcagttttgacgcgaagttcgagcaactcgcctgtcatttctcggcgtttgtttgcttccgctaatcgctgtcgcgtctcctgcgcatacttactttctgggtcagcccatctgcgtgcattcgatgtagctgcgccccgtcgccccatcgtcgctagagctttccgccctcggctgctctgcgtttccacccgacgagcagggacgactggctggcctttagccacgtagccgcgcacacgacgcgccatcgtcaggcgatcacgcatggcgggaagatccggctcccggccgtctgcaccgaccgcctgggcaacgttgtacgccacttcatacgcgtcgatgatcttggcatcttttaggcgctcaccagcagctttgagctggtatcccacggtcaacgcgtggcgaaacgcggtctcgtcgcgcgctcgctctggatttgtccagagcactcgcacgccgtcgatcaggtcgccggacgcgtccagggcgctcggcaggctcgcgtccaaaatcgctagcgccttggcttctgcggtggcgcgttgtgccgcttcaatgcgggcgcgtccgctggaaaagtcctgctcaatgtactttttcggcttctgtgatccggtcatcgttcgagcaatctccattaggtcggccagccgatccacacgatcatgctggcagtgccatttataggctgtcggatcgtctgagacgtgcagcggccaccggctcagcctatgcgaaaaagcctggtcagcgccgaaaacacgagtcatttcttccgtcgttgcagccagcaggcgcatatttgggctggttttacctgctgcggcatacaccgggtcaatgagccagatgagctggcatttcccgctcagcggattcacgccgatccaagccggcgctttttctaggcgtgcccatttctctaaaatcgcgtagacctgcgggtttacgtgctcaatcttcccgccggcctggtggctgggcacatcgatgtcaagcacgatcaccgcggcatgttgcgcgtgcgtcagcgcaacgtactggcaccgcgtcagcgcttttgagccagcccggtagagctttggttgggtttcgccggtatccgggtttttaatccaggcgctcgcgaaatctcttgtcttgctgccctggaagctttcgcgtcccaggtgagcgagcagttcgcggcgatcttctgccgtccagccgcgtgagccgcagcgcatagcttcggggtgggtgtcgaacagatcggcggacaatttccacgcgctagctgtgactgtgtcctgcggatcggctagagtcatgtcttgagtgctttctcccagctgatgactgggggttagccgacgccctgtgagttcccgctcacggggcgttcaactttttcaggtatttgtgcagcttatcgtgttttcttcgtaaatgaacgcttaactaccttgttaaacgtggcaaataggcaggattgatggggatctagcttcacgctgccgcaagcactcagggcgcaagggctgctaaaggaagcggaacacgtagaaagccagtccgcagaaacggtgctgaccccggatgaatgtcagctactgggctatctggacaagggaaaacgcaagcgcaaagagaaagcaggtagcttgcagtgggcttacatggcgatagctagactgggcggttttatggacagcaagcgaaccggaattgccagctggggcgccctctggtaaggttgggaagccctgcaaagtaaactggatggctttcttgccgccaaggatctgatggcgcaggggatcaagatctgatcaagagacaggatgaggatcgtttcgcatgattgaacaagatggattgcacgcaggttctccggccgcttgggtggagaggctattcggctatgactgggcacaacagacaatcggctgctctgatgccgccgtgttccggctgtcagcgcaggggcgcccggttctttttgtcaagaccgacctgtccggtgccctgaatgaactccaagacgaggcagcgcggctatcgtggctggccacgacgggcgttccttgcgcagctgtgctcgacgttgtcactgaagcgggaagggactggctgctattgggcgaagtgccggggcaggatctcctgtcatctcaccttgctcctgccgagaaagtatccatcatggctgatgcaatgcggcggctgcatacgcttgatccggctacctgcccattcgaccaccaagcgaaacatcgcatcgagcgagcacgtactcggatggaagccggtcttgtcgatcaggatgatctggacgaagagcatcaggggctcgcgccagccgaactgttcgccaggctcaaggcgcggatgcccgacggcgaggatctcgtcgtgacccatggcgatgcctgcttgccgaatatcatggtggaaaatggccgcttttctggattcatcgactgtggccggctgggtgtggcggaccgctatcaggacatagcgttggctacccgtgatattgctgaagagcttggcggcgaatgggctgaccgcttcctcgtgctttacggtatcgccgctcccgattcgcagcgcatcgccttctatcgccttcttgacgagttcttctgagcgggactctggggttcgcggaatcatgaccaaaatcccttaacgtgagttttcgttccactgagcgtcagaccccgtagaaaagatcaaaggatcttcttgagatcctttttttctgcgcgtaatctgctgcttgcaaacaaaaaaaccaccgctaccagcggtggtttgtttgccggatcaagagctaccaactctttttccgaaggtaactggcttcagcagagcgcagataccaaatactgtccttctagtgtagccgtagttaggccaccacttcaagaactctgtagcaccgcctacatacctcgctctgctaatcctgttaccagtggctgctgccagtggcgataagtcgtgtcttaccgggttggactcaagacgatagttaccggataaggcgcagcggtcgggctgaacggggggttcgtgcacacagcccagcttggagcgaacgacctacaccgaactgagatacctacagcgtgagctatgagaaagcgccacgcttcccgaagggagaaaggcggacaggtatccggtaagcggcagggtcggaacaggagagcgcacgagggagcttccagggggaaacgcctggtatctttatagtcctgtcgggtttcgccacctctgacttgagcgtcgatttttgtgatgctcgtcaggggggcggagcctatggaaaaacgccagcaacgcggcctttttacggttcctggccttttgctggccttttgctcacatgttctttcctgcgttatcccctgattctgtggataaccgtattaccgcctttgagtgagctgataccgctcgccgcagccgaacgaccgagcgcagcgagtcagtgagcgaggaagcggaagagtgcctgatgcggtattttctccttacgcatctgtgcggtatttcacaccg

SEQ ID NO: 6 - DNA, 78 bp, Artificial Sequence
  引物序列
gcgctcacaatttcacacaggaaacagaattaattaagcttaaaggcacccgatatggataagaaatactcaataggc

SEQ ID NO: 7 - DNA, 27 bp, Artificial Sequence
  引物序列
tcagtcacctcctagctgactcaaatc

SEQ ID NO: 8 - DNA, 42 bp, Artificial Sequence
  引物序列
gtcagctaggaggtgactgaagcttggctgttttggcggatg

SEQ ID NO: 9 - DNA, 30 bp, Artificial Sequence
  引物序列
ctgtgtgaaattgtgagcgctcacaattcc

SEQ ID NO: 10 - DNA, 42 bp, Artificial Sequence
  引物序列
ctgtgcggtatttcacaccggtgcgtggcgagttttacaaag

SEQ ID NO: 11 - DNA, 82 bp, Artificial Sequence
  引物序列
gttcttgtaatcctccaaaattgtggtggcactgtcctggtcgagcttaccaccttttgtacttagatgatgattcagggac

SEQ ID NO: 12 - DNA, 43 bp, Artificial Sequence
  引物序列
ttttggaggattacaagaacatgactaagcaaccaccaatcgc

SEQ ID NO: 13 - DNA, 25 bp, Artificial Sequence
  引物序列
ttcctctgaattatcgattacactg

SEQ ID NO: 14 - DNA, 45 bp, Artificial Sequence
  引物序列
taatcgataattcagaggaataactgttttggcggatgagagaag

SEQ ID NO: 15 - DNA, 23 bp, Artificial Sequence
  引物序列
ggagacctttttggagctagtcg

SEQ ID NO: 16 - DNA, 23 bp, Artificial Sequence
  引物序列
ctagctccaaaaaggtctccagg

SEQ ID NO: 17 - DNA, 23 bp, Artificial Sequence
  引物序列
cggtgtgaaataccgcacagatg

SEQ ID NO: 18 - DNA, 24 bp, Artificial Sequence
  引物序列
ttcatgcagaaatcaacattgaca

SEQ ID NO: 19 - DNA, 24 bp, Artificial Sequence
  引物序列
aaactgtcaatgttgatttctgca

SEQ ID NO: 20 - DNA, 24 bp, Artificial Sequence
  引物序列
ttcagcaggtgaaggtgatgtcgg

SEQ ID NO: 21 - DNA, 24 bp, Artificial Sequence
  引物序列
aaacccgacatcaccttcacctgc

SEQ ID NO: 22 - DNA, 90 bp, Artificial Sequence
  引物序列
ggtggtgccgtcttctacagaagagacgttctgcagaaccatgtcgargttgatttctgcatcagccaacgcacggaaaaccttcgcagc

SEQ ID NO: 23 - DNA, 90 bp, Artificial Sequence
  引物序列
ggtggtgccgtcttctacagaagagacgttctgcagaaccatgtccwtgttgatttctgcatcagccaacgcacggaaaaccttcgcagc

SEQ ID NO: 24 - DNA, 90 bp, Artificial Sequence
  引物序列
ggtggtgccgtcttctacagaagagacgttctgcagaaccatgtcgghgttgatttctgcatcagccaacgcacggaaaaccttcgcagc

SEQ ID NO: 25 - DNA, 90 bp, Artificial Sequence
  引物序列
ggtggtgccgtcttctacagaagagacgttctgcagaaccatgtcgtdgttgatttctgcatcagccaacgcacggaaaaccttcgcagc

SEQ ID NO: 26 - DNA, 90 bp, Artificial Sequence
  引物序列
ggtggtgccgtcttctacagaagagacgttctgcagaaccatgtctkggttgatttctgcatcagccaacgcacggaaaaccttcgcagc

SEQ ID NO: 27 - DNA, 90 bp, Artificial Sequence
  引物序列
ggtggtgccgtcttctacagaagagacgttctgcagaaccatgtcwtcgttgatttctgcatcagccaacgcacggaaaaccttcgcagc

SEQ ID NO: 28 - DNA, 90 bp, Artificial Sequence
  引物序列
ggtggtgccgtcttctacagaagagacgttctgcagaaccatgtcgcvgttgatttctgcatcagccaacgcacggaaaaccttcgcagc

SEQ ID NO: 29 - DNA, 90 bp, Artificial Sequence
  引物序列
ggtggtgccgtcttctacagaagagacgttctgcagaaccatgtcgacgttgatttctgcatcagccaacgcacggaaaaccttcgcagc

SEQ ID NO: 30 - DNA, 90 bp, Artificial Sequence
  引物序列
ggtggtgccgtcttctacagaagagacgttctgcagaaccatgtcccagttgatttctgcatcagccaacgcacggaaaaccttcgcagc

SEQ ID NO: 31 - DNA, 90 bp, Artificial Sequence
  引物序列
gtcggtggtgccgtcttctacagaagagacgttctgcagaaccatgadaatgttgatttctgcatcagccaacgcacggaaaaccttcgc

SEQ ID NO: 32 - DNA, 90 bp, Artificial Sequence
  引物序列
gtcggtggtgccgtcttctacagaagagacgttctgcagaaccatcwtaatgttgatttctgcatcagccaacgcacggaaaaccttcgc

SEQ ID NO: 33 - DNA, 90 bp, Artificial Sequence
  引物序列
gtcggtggtgccgtcttctacagaagagacgttctgcagaaccatgghaatgttgatttctgcatcagccaacgcacggaaaaccttcgc

SEQ ID NO: 34 - DNA, 90 bp, Artificial Sequence
  引物序列
gtcggtggtgccgtcttctacagaagagacgttctgcagaaccatgtdaatgttgatttctgcatcagccaacgcacggaaaaccttcgc

SEQ ID NO: 35 - DNA, 90 bp, Artificial Sequence
  引物序列
gtcggtggtgccgtcttctacagaagagacgttctgcagaaccattkgaatgttgatttctgcatcagccaacgcacggaaaaccttcgc

SEQ ID NO: 36 - DNA, 90 bp, Artificial Sequence
  引物序列
gtcggtggtgccgtcttctacagaagagacgttctgcagaaccatttcaatgttgatttctgcatcagccaacgcacggaaaaccttcgc

SEQ ID NO: 37 - DNA, 90 bp, Artificial Sequence
  引物序列
gtcggtggtgccgtcttctacagaagagacgttctgcagaaccatgcvaatgttgatttctgcatcagccaacgcacggaaaaccttcgc

SEQ ID NO: 38 - DNA, 90 bp, Artificial Sequence
  引物序列
gtcggtggtgccgtcttctacagaagagacgttctgcagaaccatgacaatgttgatttctgcatcagccaacgcacggaaaaccttcgc

SEQ ID NO: 39 - DNA, 90 bp, Artificial Sequence
  引物序列
gtcggtggtgccgtcttctacagaagagacgttctgcagaaccatccaaatgttgatttctgcatcagccaacgcacggaaaaccttcgc

SEQ ID NO: 40 - DNA, 90 bp, Artificial Sequence
  引物序列
cgcgcggcggccgtcggaacgagggcaggtgaaggtgatgtcggtgadgccgtcttctacagaagagacgttctgcagaaccatgtcaat

SEQ ID NO: 41 - DNA, 90 bp, Artificial Sequence
  引物序列
cgcgcggcggccgtcggaacgagggcaggtgaaggtgatgtcggtcwtgccgtcttctacagaagagacgttctgcagaaccatgtcaat

SEQ ID NO: 42 - DNA, 90 bp, Artificial Sequence
  引物序列
cgcgcggcggccgtcggaacgagggcaggtgaaggtgatgtcggtagmgccgtcttctacagaagagacgttctgcagaaccatgtcaat

SEQ ID NO: 43 - DNA, 90 bp, Artificial Sequence
  引物序列
cgcgcggcggccgtcggaacgagggcaggtgaaggtgatgtcggtgtdgccgtcttctacagaagagacgttctgcagaaccatgtcaat

SEQ ID NO: 44 - DNA, 90 bp, Artificial Sequence
  引物序列
cgcgcggcggccgtcggaacgagggcaggtgaaggtgatgtcggttkggccgtcttctacagaagagacgttctgcagaaccatgtcaat

SEQ ID NO: 45 - DNA, 90 bp, Artificial Sequence
  引物序列
cgcgcggcggccgtcggaacgagggcaggtgaaggtgatgtcggtwtcgccgtcttctacagaagagacgttctgcagaaccatgtcaat

SEQ ID NO: 46 - DNA, 90 bp, Artificial Sequence
  引物序列
cgcgcggcggccgtcggaacgagggcaggtgaaggtgatgtcggtgcvgccgtcttctacagaagagacgttctgcagaaccatgtcaat

SEQ ID NO: 47 - DNA, 90 bp, Artificial Sequence
  引物序列
cgcgcggcggccgtcggaacgagggcaggtgaaggtgatgtcggtgacgccgtcttctacagaagagacgttctgcagaaccatgtcaat

SEQ ID NO: 48 - DNA, 90 bp, Artificial Sequence
  引物序列
cgcgcggcggccgtcggaacgagggcaggtgaaggtgatgtcggtccagccgtcttctacagaagagacgttctgcagaaccatgtcaat

SEQ ID NO: 49 - DNA, 22 bp, Artificial Sequence
  引物序列
cggacgttgacggtgtgtatac

SEQ ID NO: 50 - DNA, 23 bp, Artificial Sequence
  引物序列
gcacggaaatacgaatctcagag